European Patent Application EP 4 501 941 A1, published February 5, 2025. Title: Peptide Compound which shows TrkB binding activity. Applicant: PeptiDream INC. The sequence listing filed with the application follows.

SEQUENCE LISTING (41 sequences)

SEQ ID NO: 1 - skipped

SEQ ID NO: 2 - protein, 15 aa, synthetic construct
  REGION 1..15: note = Synthesized polypeptide
  SITE 5: note = MISC_FEATURE - Xaa is 3Py
  SITE 12: note = MISC_FEATURE - Xaa is 3Py
FLPYXWPTYSLXVWC

SEQ ID NO: 3 - protein, 16 aa, synthetic construct
  REGION 1..16: note = Synthesized polypeptide
  SITE 5: note = MISC_FEATURE - Xaa is 3Py
  SITE 12: note = MISC_FEATURE - Xaa is 3Py
FLPYXWPTYSLXVWCG

SEQ ID NO: 4 - protein, 16 aa, synthetic construct
  REGION 1..16: note = Synthesized polypeptide
  SITE 5: note = MISC_FEATURE - Xaa is 3Py
  SITE 12: note = MISC_FEATURE - Xaa is 3Py
FEPYXWPTYSLXVWCG

SEQ ID NO: 5 - protein, 16 aa, synthetic construct
  REGION 1..16: note = Synthesized polypeptide
  SITE 5: note = MISC_FEATURE - Xaa is 3Py
  SITE 12: note = MISC_FEATURE - Xaa is 3Py
FSPYXWPTYSLXVWCG

SEQ ID NO: 6 - protein, 16 aa, synthetic construct
  REGION 1..16: note = Synthesized polypeptide
  SITE 5: note = MISC_FEATURE - Xaa is 3Py
  SITE 12: note = MISC_FEATURE - Xaa is 3Py
FLPYXWPTYSEXVWCG

SEQ ID NO: 7 - protein, 16 aa, synthetic construct
  REGION 1..16: note = Synthesized polypeptide
  SITE 5: note = MISC_FEATURE - Xaa is 3Py
  SITE 12: note = MISC_FEATURE - Xaa is 3Py
FLPYXWPTYSLXVPCG

SEQ ID NO: 8 - protein, 16 aa, synthetic construct
  REGION 1..16: note = Synthesized polypeptide
  SITE 5: note = MISC_FEATURE - Xaa is 3Py
  SITE 12: note = MISC_FEATURE - Xaa is 3Py
FLPYXWPTYSLXVYCG

SEQ ID NO: 9 - protein, 16 aa, synthetic construct
  REGION 1..16: note = Synthesized polypeptide
  SITE 5: note = MISC_FEATURE - Xaa is 3Py
  SITE 12: note = MISC_FEATURE - Xaa is 3Py
FLPYXWPTYSLXVSCG

SEQ ID NO: 10 - protein, 16 aa, synthetic construct
  REGION 1..16: note = Synthesized polypeptide
  SITE 5: note = MISC_FEATURE - Xaa is 3Py
  SITE 12: note = MISC_FEATURE - Xaa is 3Py
FLPYXWPTYSLXVACG

SEQ ID NO: 11 - protein, 16 aa, synthetic construct
  REGION 1..16: note = Synthesized polypeptide
  SITE 5: note = MISC_FEATURE - Xaa is 3Py
  SITE 12: note = MISC_FEATURE - Xaa is 3Py
FLPYXWPTYSLXVECG

SEQ ID NO: 12 - protein, 16 aa, synthetic construct
  REGION 1..16: note = Synthesized polypeptide
  SITE 5: note = MISC_FEATURE - Xaa is 3Py
  SITE 12: note = MISC_FEATURE - Xaa is 3Py
FSPYXWPTYSEXVWCG

SEQ ID NO: 13 - protein, 16 aa, synthetic construct
  REGION 1..16: note = Synthesized polypeptide
  SITE 5: note = MISC_FEATURE - Xaa is 3Py
  SITE 12: note = MISC_FEATURE - Xaa is 3Py
FSPYXWPTYSLXVECG

SEQ ID NO: 14 - protein, 16 aa, synthetic construct
  REGION 1..16: note = Synthesized polypeptide
  SITE 5: note = MISC_FEATURE - Xaa is 3Py
  SITE 12: note = MISC_FEATURE - Xaa is 3Py
FLPYXWPTYSEXVECG

SEQ ID NO: 15 - protein, 16 aa, synthetic construct
  REGION 1..16: note = Synthesized polypeptide
  SITE 5: note = MISC_FEATURE - Xaa is 3Py
  SITE 12: note = MISC_FEATURE - Xaa is 3Py
FSPYXWPTYSEXVECG

SEQ ID NO: 16 - protein, 16 aa, synthetic construct
  REGION 1..16: note = Synthesized polypeptide
  SITE 5: note = MISC_FEATURE - Xaa is 3Py
  SITE 12: note = MISC_FEATURE - Xaa is 3Py
FEPYXWPTYSLXVSCG

SEQ ID NO: 17 - protein, 16 aa, synthetic construct
  REGION 1..16: note = Synthesized polypeptide
  SITE 5: note = MISC_FEATURE - Xaa is 3Py
  SITE 12: note = MISC_FEATURE - Xaa is 3Py
FEPYXWPTYSEXVECG

SEQ ID NO: 18 - protein, 16 aa, synthetic construct
  REGION 1..16: note = Synthesized polypeptide
  SITE 5: note = MISC_FEATURE - Xaa is 3Py
  SITE 12: note = MISC_FEATURE - Xaa is 3Py
FEPYXWPTYSEXVSCG

SEQ ID NO: 19 - protein, 16 aa, synthetic construct
  REGION 1..16: note = Synthesized polypeptide
  SITE 5: note = MISC_FEATURE - Xaa is 3Py
  SITE 12: note = MISC_FEATURE - Xaa is 4Py
FSPYXWPSYSLXVECG

SEQ ID NO: 20 - protein, 16 aa, synthetic construct
  REGION 1..16: note = Synthesized polypeptide
  SITE 5: note = MISC_FEATURE - Xaa is 3Py
  SITE 7: note = MISC_FEATURE - Xaa is P4Sh
  SITE 12: note = MISC_FEATURE - Xaa is 4Py
FSPYXWXSYSLXVECG

SEQ ID NO: 21 - protein, 16 aa, synthetic construct
  REGION 1..16: note = Synthesized polypeptide
  SITE 3: note = MISC_FEATURE - Xaa is P4Sh
  SITE 5: note = MISC_FEATURE - Xaa is 3Py
  SITE 7: note = MISC_FEATURE - Xaa is P4Sh
  SITE 12: note = MISC_FEATURE - Xaa is 4Py
FSXYXWXSYSLXVECG

SEQ ID NO: 22 - protein, 16 aa, synthetic construct
  REGION 1..16: note = Synthesized polypeptide
  SITE 5: note = MISC_FEATURE - Xaa is 3Py
  SITE 7: note = MISC_FEATURE - Xaa is P4Sh
  SITE 12: note = MISC_FEATURE - Xaa is 4Py
FDPYXWXSYSLXVECG

SEQ ID NO: 23 - protein, 16 aa, synthetic construct
  REGION 1..16: note = Synthesized polypeptide
  SITE 4: note = MISC_FEATURE - Xaa is F4COO
  SITE 5: note = MISC_FEATURE - Xaa is 3Py
  SITE 7: note = MISC_FEATURE - Xaa is P4Sh
  SITE 12: note = MISC_FEATURE - Xaa is 4Py
FSPXXWXSYSLXVECG

SEQ ID NO: 24 - protein, 16 aa, synthetic construct
  REGION 1..16: note = Synthesized polypeptide
  SITE 3: note = MISC_FEATURE - Xaa is P4Sh
  SITE 4: note = MISC_FEATURE - Xaa is F4COO
  SITE 5: note = MISC_FEATURE - Xaa is 3Py
  SITE 7: note = MISC_FEATURE - Xaa is P4Sh
  SITE 12: note = MISC_FEATURE - Xaa is 4Py
FSXXXWXSYSLXVECG

SEQ ID NO: 25 - protein, 16 aa, synthetic construct
  REGION 1..16: note = Synthesized polypeptide
  SITE 3: note = MISC_FEATURE - Xaa is P4Sh
  SITE 4: note = MISC_FEATURE - Xaa is F4COO
  SITE 5: note = MISC_FEATURE - Xaa is 3Py
  SITE 7: note = MISC_FEATURE - Xaa is P4Sh
  SITE 12: note = MISC_FEATURE - Xaa is 4Py
FDXXXWXSYSLXVECG

SEQ ID NO: 26 - protein, 16 aa, synthetic construct
  REGION 1..16: note = Synthesized polypeptide
  SITE 5: note = MISC_FEATURE - Xaa is 3Py
  SITE 12: note = MISC_FEATURE - Xaa is 3Py
FQPYXWPTYSLXVECG

SEQ ID NO: 27 - protein, 16 aa, synthetic construct
  REGION 1..16: note = Synthesized polypeptide
  SITE 2: note = MISC_FEATURE - Xaa is Cit
  SITE 5: note = MISC_FEATURE - Xaa is 3Py
  SITE 12: note = MISC_FEATURE - Xaa is 3Py
FXPYXWPTYSLXVECG

SEQ ID NO: 28 - protein, 16 aa, synthetic construct
  REGION 1..16: note = Synthesized polypeptide
  SITE 5: note = MISC_FEATURE - Xaa is 3Py
  SITE 10: note = MISC_FEATURE - Xaa is SMe
  SITE 12: note = MISC_FEATURE - Xaa is 3Py
FSPYXWPTYXLXVECG

SEQ ID NO: 29 - protein, 16 aa, synthetic construct
  REGION 1..16: note = Synthesized polypeptide
  SITE 5: note = MISC_FEATURE - Xaa is 3Py
  SITE 12: note = MISC_FEATURE - Xaa is 3Py
FLPYXWPTYSEXVECG

SEQ ID NO: 30 - protein, 16 aa, synthetic construct
  REGION 1..16: note = Synthesized polypeptide
  SITE 1: note = MISC_FEATURE - Xaa is 4Py
  SITE 5: note = MISC_FEATURE - Xaa is 3Py
  SITE 12: note = MISC_FEATURE - Xaa is 3Py
XLPYXWPTYSEXVECG

SEQ ID NO: 31 - protein, 16 aa, synthetic construct
  REGION 1..16: note = Synthesized polypeptide
  SITE 5: note = MISC_FEATURE - Xaa is 3Py
  SITE 12: note = MISC_FEATURE - Xaa is 3Py
FQPYXWPTYSEXVECG

SEQ ID NO: 32 - protein, 16 aa, synthetic construct
  REGION 1..16: note = Synthesized polypeptide
  SITE 2: note = MISC_FEATURE - Xaa is Cit
  SITE 5: note = MISC_FEATURE - Xaa is 3Py
  SITE 12: note = MISC_FEATURE - Xaa is 3Py
FXPYXWPTYSEXVECG

SEQ ID NO: 33 - protein, 16 aa, synthetic construct
  REGION 1..16: note = Synthesized polypeptide
  SITE 4: note = MISC_FEATURE - Xaa is F4CON
  SITE 5: note = MISC_FEATURE - Xaa is 3Py
  SITE 12: note = MISC_FEATURE - Xaa is 3Py
FLPXXWPTYSEXVECG

SEQ ID NO: 34 - protein, 16 aa, synthetic construct
  REGION 1..16: note = Synthesized polypeptide
  SITE 5: note = MISC_FEATURE - Xaa is 3Py
  SITE 11: note = MISC_FEATURE - Xaa is Hgl
  SITE 12: note = MISC_FEATURE - Xaa is 3Py
FLPYXWPTYSXXVECG

SEQ ID NO: 35 - protein, 16 aa, synthetic construct
  REGION 1..16: note = Synthesized polypeptide
  SITE 5: note = MISC_FEATURE - Xaa is 3Py
  SITE 11: note = MISC_FEATURE - Xaa is Atp
  SITE 12: note = MISC_FEATURE - Xaa is 3Py
FLPYXWPTYSXXVECG

SEQ ID NO: 36 - protein, 16 aa, synthetic construct
  REGION 1..16: note = Synthesized polypeptide
  SITE 5: note = MISC_FEATURE - Xaa is 3Py
  SITE 11: note = MISC_FEATURE - Xaa is KAc
  SITE 12: note = MISC_FEATURE - Xaa is 3Py
FLPYXWPTYSXXVECG

SEQ ID NO: 37 - protein, 16 aa, synthetic construct
  REGION 1..16: note = Synthesized polypeptide
  SITE 5: note = MISC_FEATURE - Xaa is 3Py
  SITE 11: note = MISC_FEATURE - Xaa is A4paa
  SITE 12: note = MISC_FEATURE - Xaa is 3Py
FLPYXWPTYSXXVECG

SEQ ID NO: 38 - protein, 16 aa, synthetic construct
  REGION 1..16: note = Synthesized polypeptide
  SITE 5: note = MISC_FEATURE - Xaa is 3Py
  SITE 10: note = MISC_FEATURE - Xaa is SMe
  SITE 12: note = MISC_FEATURE - Xaa is 3Py
FSPYXWPTYXEXVECG

SEQ ID NO: 39 - protein, 16 aa, synthetic construct
  REGION 1..16: note = Synthesized polypeptide
  SITE 5: note = MISC_FEATURE - Xaa is 3Py
  SITE 10: note = MISC_FEATURE - Xaa is SMe
  SITE 12: note = MISC_FEATURE - Xaa is 3Py
FQPYXWPTYXEXVECG

SEQ ID NO: 40 - protein, 16 aa, synthetic construct
  REGION 1..16: note = Synthesized polypeptide
  SITE 5: note = MISC_FEATURE - Xaa is 3Py
  SITE 11: note = MISC_FEATURE - Xaa is Hgl
  SITE 12: note = MISC_FEATURE - Xaa is 3Py
FQPYXWPTYSXXVECG

SEQ ID NO: 41 - protein, 16 aa, synthetic construct
  REGION 1..16: note = Synthesized polypeptide
  SITE 1: note = MISC_FEATURE - Xaa is 4Py
  SITE 3: note = MISC_FEATURE - Xaa is P4Sh
  SITE 4: note = MISC_FEATURE - Xaa is F4CON
  SITE 5: note = MISC_FEATURE - Xaa is 3Py
  SITE 10: note = MISC_FEATURE - Xaa is SMe
  SITE 11: note = MISC_FEATURE - Xaa is A4paa
  SITE 12: note = MISC_FEATURE - Xaa is 4Py
XQXXXWPSYXXXVECG